European Patent Specification EP 3 805 380 B1, published December 3, 2025. Title: IMPROVED THERMOSTABLE VIRAL REVERSE TRANSCRIPTASE. Applicant: Qiagen Beverly, LLC. The sequence listing filed with the application follows.

SEQUENCE LISTING (14 sequences)

SEQ ID NO: 1 - DNA, 1674 bp, Artificial Sequence
  source 1..1674: /mol_type="unassigned DNA" /note="Synthetic gene" /organism="Artificial Sequence"
atggcacagctgagcaaagaaatcaaatttcgcaaaatcgaactgaaagaaggcaccatgggtccgaaaattccgcagtggcctctgaccaaagaaaaactggaaggtgcaaaagaaattgttcagcgtctgctgagcgaaggtaaaattagcgaagcaagcgataataacccgtataacagcccgattttcgtgatcaaaaaacgtagcggtaaatggcgtctgctgcaggatctgcgtgaactgaataaaaccgttcaggttggcaccgaaattagccgtggtctgccgcatccgggtggtctgattaaatgtaaacacatgaccgttctggatattggcgacgcatattttaccattccgctggatccggaatttcgtccgtataccgcatttacaattccgagcattaatcatcaagaaccggataaacgttatgtgtggaattgcctgccgcagggttttgttctgagcccgtatatctatcagaaaacgctgcaagaaattctgcagccatttcgtgaacgttatccggaagttcagctgtatcagtatatggatgacctgtttgtgggtagcaatggtagcaaaaaacagcacaaagaactgatcattgaactgcgtgcaattctgctggaaaaaggttttgaaacaccggatgataaactgcaagaagttccgccttatagctggctgggttatcagctgtgtccggaaaattggaaagttcagaaaatgcagctggatatggttaaaaatccgaccctgaatgatgtgcagaaactgatgggcaatattacctggatgagcagcggtgttccgggtctgaccgttaaacatattgcagcaaccaccaaaggttgtctggaactgaatcagaaagttatctggaccgaagaagcacaaaaagaactggaagaaaacaacgagaaaatcaaaaatgcacagggcctgcagtattataacccggaagaagaaatgctttgcgaagtggaaatcaccaaaaactatgaagccacctatgtgattaaacagagccagggtattctgtgggcaggcaaaaaaatcatgaaagccaataaaggttggagcaccgtgaaaaatctgatgctgctgctgcaacatgtggcaaccgaaagcattacccgtgttggtaaatgtccgacctttaaagttccgtttaccaaagaacaggtgatgtgggaaatgcagaaaggttggtattatagttggctgccggaaattgtttatacccatcaggttgttcatgatgactggcgtatgaaactggttgaagaaccgaccagcggtattaccatttataccgatggtggtaaacagaatggtgaaggtattgcagcctatgttaccagcaatggtcgtaccaaacagaaacgtctgggtccggttacacatcaggtggcagaacgtatggcaattcagatggcactggaagatacccgtgataaacaggttaatattgtgaccgatagctattattgttggaaaaacattaccgaaggtctgggtctggaaggtccgcagagcccgtggtggccgattattcagaatattcgcgaaaaagaaatcgtgtactttgcatgggttccaggtcataaaggtatttgtggtaatcagctggcagatgaagcagccaaaatcaaagaagagatc

SEQ ID NO: 2 - protein, 558 aa, Artificial Sequence
  Expression from a synthetic gene
MAQLSKEIKFRKIELKEGTMGPKIPQWPLTKEKLEGAKEIVQRLLSEGKISEASDNNPYNSPIFVIKKRSGKWRLLQDLRELNKTVQVGTEISRGLPHPGGLIKCKHMTVLDIGDAYFTIPLDPEFRPYTAFTIPSINHQEPDKRYVWNCLPQGFVLSPYIYQKTLQEILQPFRERYPEVQLYQYMDDLFVGSNGSKKQHKELIIELRAILLEKGFETPDDKLQEVPPYSWLGYQLCPENWKVQKMQLDMVKNPTLNDVQKLMGNITWMSSGVPGLTVKHIAATTKGCLELNQKVIWTEEAQKELEENNEKIKNAQGLQYYNPEEEMLCEVEITKNYEATYVIKQSQGILWAGKKIMKANKGWSTVKNLMLLLQHVATESITRVGKCPTFKVPFTKEQVMWEMQKGWYYSWLPEIVYTHQVVHDDWRMKLVEEPTSGITIYTDGGKQNGEGIAAYVTSNGRTKQKRLGPVTHQVAERMAIQMALEDTRDKQVNIVTDSYYCWKNITEGLGLEGPQSPWWPIIQNIREKEIVYFAWVPGHKGICGNQLADEAAKIKEEI

SEQ ID NO: 3 - DNA, 1674 bp, Artificial Sequence
  source 1..1674: /mol_type="unassigned DNA" /note="Synthetic gene" /organism="Artificial Sequence"
atggcacagctgagcaaagaaatcaaatttcgcaaaatcgaactgaaagaaggcaccatgggtccgaaaattccgcagtggcctctgaccaaagaaaaactggaaggtgcaaaagaaattgttcagcgtctgctgagcgaaggtaaaattagcgaagcaagcgataataacccgtataacagcccgattttcgtgatcaaaaaacgtagcggtaaatggcgtctgctgcaggatctgcgtgaactgaataaaaccgttcaggttggcaccgaaattagccgtggtctgccgcatccgggtggtctgattaaatgtaaacacatgaccgttctggatattggcgacgcatattttaccattccgctggatccggaatttcgtccgtataccgcatttacaattccgagcattaatcatcaagaaccggataaacgttatgtgtggaattgcctgccgcagggttttgttctgagcccgtatatctatcagaaaacgctgcaagaaattctgcagccatttcgtgaacgttatccggaagttcagctgtatcagtatatggatgacctgtttgtgggtagcaatggtagcaaaaaacagcacaaagaactgatcattgaactgcgtgcaattctgctggaaaaaggttttgaaacaccggatgataaactgcaagaagttccgccttatagctggctgggttatcagctgtgtccggaaaattggaaagttcagaaaatgcagctggatatggttaaaaatccgaccctgaatgatgtgcagaaactgatgggcaatattacctggatgagcagcggtgttccgggtctgaccgttaaacatattgcagcaaccaccaaaggttgtctggaactgaatcagaaagttatctggaccgaagaagcacaaaaagaactggaagaaaacaacgagaaaatcaaaaatgcacagggcctgcagtattataacccggaagaagaaatgctttgcgaagtggaaatcaccaaaaactatgaagccacctatgtgattaaacagagccagggtattctgtgggcaggcaaaaaaatcatgaaagccaataaaggttggagcaccgtgaaaaatctgatgctgctgctgcaacatgtggcaaccgaaagcattacccgtgttggtaaatgtccgacctttaaagttccgtttaccaaagaacaggtgatgtgggaaatgcagaaaggttggtattatagttggctgccggaaattgtttatacccatcaggttgttcatgatgactggcgtatgaaactggttgaagaaccgaccagcggtattaccatttataccggtggtggtaaacagaatggtgaaggtattgcagcctatgttaccagcaatggtcgtaccaaacagaaacgtctgggtccggttacacatcaggtggcagaacgtatggcaattcagatggcactggaagatacccgtgataaacaggttaatattgtgaccgatagctattattgttggaaaaacattaccgaaggtctgggtctggaaggtccgcagagcccgtggtggccgattattcagaatattcgcgaaaaagaaatcgtgtactttgcatgggttccaggtcataaaggtatttgtggtaatcagctggcagatgaagcagccaaaatcaaagaagagatc

SEQ ID NO: 4 - protein, 558 aa, Artificial Sequence
  Expression from a synthetic gene
MAQLSKEIKFRKIELKEGTMGPKIPQWPLTKEKLEGAKEIVQRLLSEGKISEASDNNPYNSPIFVIKKRSGKWRLLQDLRELNKTVQVGTEISRGLPHPGGLIKCKHMTVLDIGDAYFTIPLDPEFRPYTAFTIPSINHQEPDKRYVWNCLPQGFVLSPYIYQKTLQEILQPFRERYPEVQLYQYMDDLFVGSNGSKKQHKELIIELRAILLEKGFETPDDKLQEVPPYSWLGYQLCPENWKVQKMQLDMVKNPTLNDVQKLMGNITWMSSGVPGLTVKHIAATTKGCLELNQKVIWTEEAQKELEENNEKIKNAQGLQYYNPEEEMLCEVEITKNYEATYVIKQSQGILWAGKKIMKANKGWSTVKNLMLLLQHVATESITRVGKCPTFKVPFTKEQVMWEMQKGWYYSWLPEIVYTHQVVHDDWRMKLVEEPTSGITIYTGGGKQNGEGIAAYVTSNGRTKQKRLGPVTHQVAERMAIQMALEDTRDKQVNIVTDSYYCWKNITEGLGLEGPQSPWWPIIQNIREKEIVYFAWVPGHKGICGNQLADEAAKIKEEI

SEQ ID NO: 5 - DNA, 1674 bp, Artificial Sequence
  source 1..1674: /mol_type="unassigned DNA" /note="Synthetic gene" /organism="Artificial Sequence"
atggcacagctgagcaaagaaatcaaatttcgcaaaatcgaactgaaagaaggcaccatgggtccgaaaattccgcagtggcctctgaccaaagaaaaactggaaggtgcaaaagaaattgttcagcgtctgctgagcgaaggtaaaattagcgaagcaagcgataataacccgtataacagcccgattttcgtgatcaaaaaacgtagcggtaaatggcgtctgctgcaggatctgcgtgaactgaataaaaccgttcaggttggcaccgaaattagccgtggtctgccgcatccgggtggtctgattaaatgtaaacacatgaccgttctggatattggcgacgcatattttaccattccgctggatccggaatttcgtccgtataccgcatttacaattccgagcattaatcatcaagaaccggataaacgttatgtgtggaattgcctgccgcagggttttgttctgagcccgtatatctatcagaaaacgctgcaagaaattctgcagccatttcgtgaacgttatccggaagttcagctgtatcagtatatggatgacctgtttgtgggtagcaatggtagcaaaaaacagcacaaagaactgatcattgaactgcgtgcaattctgctggaaaaaggttttgaaacaccggatgataaactgcaagaagttccgccttatagctggctgggttatcagctgtgtccggaaaattggaaagttcagaaaatgcagctggatatggttaaaaatccgaccctgaatgatgtgcagaaactgatgggcaatattacctggatgagcagcggtgttccgggtctgaccgttaaacatattgcagcaaccaccaaaggttgtctggaactgaatcagaaagttatctggaccgaagaagcacaaaaagaactggaagaaaacaacgagaaaatcaaaaatgcacagggcctgcagtattataacccggaagaagaaatgctttgcgaagtggaaatcaccaaaaactatgaagccacctatgtgattaaacagagccagggtattctgtgggcaggcaaaaaaatcatgaaagccaataaaggttggagcaccgtgaaaaatctgatgctgctgctgcaacatgtggcaaccgaaagcattacccgtgttggtaaatgtccgacctttaaagttccgtttaccaaagaacaggtgatgtgggaaatgcagaaaggttggtattatagttggctgccggaaattgtttatacccatcaggttgttcatgatgactggcgtatgaaactggttgaagaaccgaccagcggtattaccatttataccggtggtggtaaacagaatggtgaaggtattgcagcctatgttaccagcaatggtcgtaccaaacagaaacgtctgggtccggttacacatcaggtggcacaacgtatggcaattcagatggcactggaagatacccgtgataaacaggttaatattgtgaccgatagctattattgttggaaaaacattaccgaaggtctgggtctggaaggtccgcagagcccgtggtggccgattattcagaatattcgcgaaaaagaaatcgtgtactttgcatgggttccaggtcataaaggtatttgtggtaatcagctggcagatgaagcagccaaaatcaaagaagagatc

SEQ ID NO: 6 - protein, 558 aa, Artificial Sequence
  Expression from a synthetic gene
MAQLSKEIKFRKIELKEGTMGPKIPQWPLTKEKLEGAKEIVQRLLSEGKISEASDNNPYNSPIFVIKKRSGKWRLLQDLRELNKTVQVGTEISRGLPHPGGLIKCKHMTVLDIGDAYFTIPLDPEFRPYTAFTIPSINHQEPDKRYVWNCLPQGFVLSPYIYQKTLQEILQPFRERYPEVQLYQYMDDLFVGSNGSKKQHKELIIELRAILLEKGFETPDDKLQEVPPYSWLGYQLCPENWKVQKMQLDMVKNPTLNDVQKLMGNITWMSSGVPGLTVKHIAATTKGCLELNQKVIWTEEAQKELEENNEKIKNAQGLQYYNPEEEMLCEVEITKNYEATYVIKQSQGILWAGKKIMKANKGWSTVKNLMLLLQHVATESITRVGKCPTFKVPFTKEQVMWEMQKGWYYSWLPEIVYTHQVVHDDWRMKLVEEPTSGITIYTGGGKQNGEGIAAYVTSNGRTKQKRLGPVTHQVAQRMAIQMALEDTRDKQVNIVTDSYYCWKNITEGLGLEGPQSPWWPIIQNIREKEIVYFAWVPGHKGICGNQLADEAAKIKEEI

SEQ ID NO: 7 - DNA, 1674 bp, Artificial Sequence
  source 1..1674: /mol_type="unassigned DNA" /note="Synthetic gene" /organism="Artificial Sequence"
atggcacagctgagcaaagaaatcaaatttcgcaaaatcgaactgaaagaaggcaccatgggtccgaaaattccgcagtggcctctgaccaaagaaaaactggaaggtgcaaaagaaattgttcagcgtctgctgagcgaaggtaaaattagcgaagcaagcgataataacccgtataacagcccgattttcgtgatcaaaaaacgtagcggtaaatggcgtctgctgcaggatctgcgtgaactgaataaaaccgttcaggttggcaccgaaattagccgtggtctgccgcatccgggtggtctgattaaatgtaaacacatgaccgttctggatattggcgacgcatattttaccattccgctggatccggaatttcgtccgtataccgcatttacaattccgagcattaatcatcaagaaccggataaacgttatgtgtggaattgcctgccgcagggttttgttctgagcccgtatatctatcagaaaacgctgcaagaaattctgcagccatttcgtgaacgttatccggaagttcagctgtatcagtatatggatgacctgtttgtgggtagcaatggtagcaaaaaacagcacaaagaactgatcattgaactgcgtgcaattctgctggaaaaaggttttgaaacaccggatgataaactgcaagaagttccgccttatagctggctgggttatcagctgtgtccggaaaattggaaagttcagaaaatgcagctggatatggttaaaaatccgaccctgaatgatgtgcagaaactggtgggcaaaattaattgggctagccagggtgttccgggtctgaccgttaaacatattgcagcaaccaccaaaggttgtctggaactgaatcagaaagttatctggaccgaagaagcacaaaaagaactggaagaaaacaacgagaaaatcaaaaatgcacagggcctgcagtattataacccggaagaagaaatgctttgcgaagtggaaatcaccaaaaactatgaagccacctatgtgattaaacagagccagggtattctgtgggcaggcaaaaaaatcatgaaagccaataaaggttggagcaccgtgaaaaatctgatgctgctgctgcaacatgtggcaaccgaaagcattacccgtgttggtaaatgtccgacctttaaagttccgtttaccaaagaacaggtgatgtgggaaatgcagaaaggttggtattatagttggctgccggaaattgtttatacccatcaggttgttcatgatgactggcgtatgaaactggttgaagaaccgaccagcggtattaccatttataccggtggtggtaaacagaatggtgaaggtattgcagcctatgttaccagcaatggtcgtaccaaacagaaacgtctgggtccggttacacatcaggtggcagaacgtatggcaattcagatggcactggaagatacccgtgataaacaggttaatattgtgaccgatagctattattgttggaaaaacattaccgaaggtctgggtctggaaggtccgcagagcccgtggtggccgattattcagaatattcgcgaaaaagaaatcgtgtactttgcatgggttccaggtcataaaggtatttgtggtaatcagctggcagatgaagcagccaaaatcaaagaagagatc

SEQ ID NO: 8 - protein, 558 aa, Artificial Sequence
  Expression from a synthetic gene
MAQLSKEIKFRKIELKEGTMGPKIPQWPLTKEKLEGAKEIVQRLLSEGKISEASDNNPYNSPIFVIKKRSGKWRLLQDLRELNKTVQVGTEISRGLPHPGGLIKCKHMTVLDIGDAYFTIPLDPEFRPYTAFTIPSINHQEPDKRYVWNCLPQGFVLSPYIYQKTLQEILQPFRERYPEVQLYQYMDDLFVGSNGSKKQHKELIIELRAILLEKGFETPDDKLQEVPPYSWLGYQLCPENWKVQKMQLDMVKNPTLNDVQKLVGKINWASQGVPGLTVKHIAATTKGCLELNQKVIWTEEAQKELEENNEKIKNAQGLQYYNPEEEMLCEVEITKNYEATYVIKQSQGILWAGKKIMKANKGWSTVKNLMLLLQHVATESITRVGKCPTFKVPFTKEQVMWEMQKGWYYSWLPEIVYTHQVVHDDWRMKLVEEPTSGITIYTGGGKQNGEGIAAYVTSNGRTKQKRLGPVTHQVAERMAIQMALEDTRDKQVNIVTDSYYCWKNITEGLGLEGPQSPWWPIIQNIREKEIVYFAWVPGHKGICGNQLADEAAKIKEEI

SEQ ID NO: 9 - DNA, 1674 bp, Artificial Sequence
  source 1..1674: /mol_type="unassigned DNA" /note="Synthetic gene" /organism="Artificial Sequence"
atggcacagctgagcaaagaaatcaaatttcgcaaaatcgaactgaaagaaggcaccatgggtccgaaaattccgcagtggcctctgaccaaagaaaaactggaaggtgcaaaagaaattgttcagcgtctgctgagcgaaggtaaaattagcgaagcaagcgataataacccgtataacagcccgattttcgtgatcaaaaaacgtagcggtaaatggcgtctgctgcaggatctgcgtgaactgaataaaaccgttcaggttggcaccgaaattagccgtggtctgccgcatccgggtggtctgattaaatgtaaacacatgaccgttctggatattggcgacgcatattttaccattccgctggatccggaatttcgtccgtataccgcatttacaattccgagcattaatcatcaagaaccggataaacgttatgtgtggaattgcctgccgcagggttttgttctgagcccgtatatctatcagaaaacgctgcaagaaattctgcagccatttcgtgaacgttatccggaagttcagctgtatcagtatatggatgacctgtttgtgggtagcaatggtagcaaaaaacagcacaaagaactgatcattgaactgcgtgcaattctgctggaaaaaggttttgaaacaccggatgataaactgcaagaagttccgccttatagctggctgggttatcagctgtgtccggaaaattggaaagttcagaaaatgcagctggatatggttaaaaatccgaccctgaatgatgtgcagaaactggtgggcaaaattaattgggctagccagggtgttccgggtctgaccgttaaacatattgcagcaaccaccaaaggttgtctggaactgaatcagaaagttatctggaccgaagaagcacaaaaagaactggaagaaaacaacgagaaaatcaaaaatgcacagggcctgcagtattataacccggaagaagaaatgctttgcgaagtggaaatcaccaaaaactatgaagccacctatgtgattaaacagagccagggtattctgtgggcaggcaaaaaaggcatgaaagccgctaaaaccaaaagcaccgtgaaaaatctgatgctgctgctgcaacatgtggcaaccgaaagcattacccgtgttggtaaatgtccgacctttaaagttccgtttaccaaagaacaggtgatgtgggaaatgcagaaaggttggtattatagttggctgccggaaattgtttatacccatcaggttgttcatgatgactggcgtatgaaactggttgaagaaccgaccagcggtattaccatttataccggtggtggtaaacagaatggtgaaggtattgcagcctatgttaccagcaatggtcgtaccaaacagaaacgtctgggtccggttacacatcaggtggcagaacgtatggcaattcagatggcactggaagatacccgtgataaacaggttaatattgtgaccgatagctattattgttggaaaaacattaccgaaggtctgggtctggaaggtccgcagagcccgtggtggccgattattcagaatattcgcgaaaaagaaatcgtgtactttgcatgggttccaggtcataaaggtatttgtggtaatcagctggcagatgaagcagccaaaatcaaagaagagatc

SEQ ID NO: 10 - protein, 558 aa, Artificial Sequence
  Expression from a synthetic gene
MAQLSKEIKFRKIELKEGTMGPKIPQWPLTKEKLEGAKEIVQRLLSEGKISEASDNNPYNSPIFVIKKRSGKWRLLQDLRELNKTVQVGTEISRGLPHPGGLIKCKHMTVLDIGDAYFTIPLDPEFRPYTAFTIPSINHQEPDKRYVWNCLPQGFVLSPYIYQKTLQEILQPFRERYPEVQLYQYMDDLFVGSNGSKKQHKELIIELRAILLEKGFETPDDKLQEVPPYSWLGYQLCPENWKVQKMQLDMVKNPTLNDVQKLVGKINWASQGVPGLTVKHIAATTKGCLELNQKVIWTEEAQKELEENNEKIKNAQGLQYYNPEEEMLCEVEITKNYEATYVIKQSQGILWAGKKGMKAAKTKSTVKNLMLLLQHVATESITRVGKCPTFKVPFTKEQVMWEMQKGWYYSWLPEIVYTHQVVHDDWRMKLVEEPTSGITIYTGGGKQNGEGIAAYVTSNGRTKQKRLGPVTHQVAERMAIQMALEDTRDKQVNIVTDSYYCWKNITEGLGLEGPQSPWWPIIQNIREKEIVYFAWVPGHKGICGNQLADEAAKIKEEI

SEQ ID NO: 11 - DNA, 1674 bp, Artificial Sequence
  source 1..1674: /mol_type="unassigned DNA" /note="Synthetic gene" /organism="Artificial Sequence"
atggcacagctgagcaaagaaatcaaatttcgcaaaatcgaactgaaagaaggcaccatgggtccgaaaattccgcagtggcctctgaccaaagaaaaactggaaggtgcaaaagaaattgttcagcgtctgctgagcgaaggtaaaattagcgaagcaagcgataataacccgtataacagcccgattttcgtgatcaaaaaacgtagcggtaaatggcgtctgctgcaggatctgcgtgaactgaataaaaccgttcaggttggcaccgaaattagccgtggtctgccgcatccgggtggtctgattaaatgtaaacacatgaccgttctggatattggcgacgcatattttaccattccgctggatccggaatttcgtccgtataccgcatttacaattccgagcattaatcatcaagaaccggataaacgttatgtgtggaattgcctgccgcagggttttgttctgagcccgtatatctatcagaaaacgctgcaagaaattctgcagccatttcgtgaacgttatccggaagttcagctgtatcagtatatggatgacctgtttgtgggtagcaatggtagcaaaaaacagcacaaagaactgatcattgaactgcgtgcaattctgctggaaaaaggttttgaaacaccggatgataaactgcaagaagttccgccttatagctggctgggttatcagctgtgtccggaaaattggaaagttcagaaaatgcagctggatatggttaaaaatccgaccctgaatgatgtgcagaaactggtgggcaaaattaattgggctagccagggtgttccgggtctgaccgttaaacatattgcagcaaccaccaaaggttgtctggaactgaatcagaaagttatctggaccgaagaagcacaaaaagaactggaagaaaacaacgagaaaatcaaaaatgcacagggcctgcagtattataacccggaagaagaaatgctttgcgaagtggaaatcaccaaaaactatgaagccacctatgtgattaaacagagccagggtattctgtgggcaggcaaaaaaatcatgaaagccaataaaggttggagcaccgtgaaaaatctgatgctgctgctgcaacatgtggcaaccgaaagcattacccgtgttggtaaatgtccgacctttaaagttccgtttaccaaagaacaggtgatgtgggaaatgcagaaaggttggtattatagttggctgccggaaattgtttatacccatcaggttgttcatgatgactggcgtatgaaactggttgaagaaccgaccagcggtattaccatttataccggtggtggtaaacagaatggtgaaggtattgcagcctatgttaccagcaatggtcgtaccaaacagaaacgtctgggtccggttacacatcaggtggcagaacgtatggcaattcagatggcactggaagatacccgtgataaacgggttaatattgtgaccgatagctattattgttggaaaaacattaccgaaggtctgggtctggaaggtccgcagagcccgtggtggccgattattcagaatattcacgaaaaagaaatcgtgtactttgcatgggttccaggtcataaaggtatttgtggtaatcagctggcagatgaagcagccaaaatcaaagaagagatc

SEQ ID NO: 12 - protein, 558 aa, Artificial Sequence
  Expression from a synthetic gene
MAQLSKEIKFRKIELKEGTMGPKIPQWPLTKEKLEGAKEIVQRLLSEGKISEASDNNPYNSPIFVIKKRSGKWRLLQDLRELNKTVQVGTEISRGLPHPGGLIKCKHMTVLDIGDAYFTIPLDPEFRPYTAFTIPSINHQEPDKRYVWNCLPQGFVLSPYIYQKTLQEILQPFRERYPEVQLYQYMDDLFVGSNGSKKQHKELIIELRAILLEKGFETPDDKLQEVPPYSWLGYQLCPENWKVQKMQLDMVKNPTLNDVQKLVGKINWASQGVPGLTVKHIAATTKGCLELNQKVIWTEEAQKELEENNEKIKNAQGLQYYNPEEEMLCEVEITKNYEATYVIKQSQGILWAGKKIMKANKGWSTVKNLMLLLQHVATESITRVGKCPTFKVPFTKEQVMWEMQKGWYYSWLPEIVYTHQVVHDDWRMKLVEEPTSGITIYTGGGKQNGEGIAAYVTSNGRTKQKRLGPVTHQVAERMAIQMALEDTRDKRVNIVTDSYYCWKNITEGLGLEGPQSPWWPIIQNIHEKEIVYFAWVPGHKGICGNQLADEAAKIKEEI

SEQ ID NO: 13 - DNA, 1674 bp, Artificial Sequence
  source 1..1674: /mol_type="unassigned DNA" /note="Synthetic gene" /organism="Artificial Sequence"
atggcacagctgagcaaagaaatcaaatttcgcaaaatcgaactgaaagaaggcaccatgggtccgaaaattccgcagtggcctctgaccaaagaaaaactggaaggtgcaaaagaaattgttcagcgtctgctgagcgaaggtaaaattagcgaagcaagcgataataacccgtataacagcccgattttcgtgatcaaaaaacgtagcggtaaatggcgtctgctgcaggatctgcgtgaactgaataaaaccgttcaggttggcaccgaaattagccgtggtctgccgcatccgggtggtctgattaaatgtaaacacatgaccgttctggatattggcgacgcatattttaccattccgctggatccggaatttcgtccgtataccgcatttacaattccgagcattaatcatcaagaaccggataaacgttatgtgtggaattgcctgccgcagggttttgttctgagcccgtatatctatcagaaaacgctgcaagaaattctgcagccatttcgtgaacgttatccggaagttcagctgtatcagtatatggatgacctgtttgtgggtagcaatggtagcaaaaaacagcacaaagaactgatcattgaactgcgtgcaattctgctggaaaaaggttttgaaacaccggatgataaactgcaagaagttccgccttatagctggctgggttatcagctgtgtccggaaaattggaaagttcagaaaatgcagctggatatggttaaaaatccgaccctgaatgatgtgcagaaactggtgggcaaaattaattgggctagccagggtgttccgggtctgaccgttaaacatattgcagcaaccaccaaaggttgtctggaactgaatcagaaagttatctggaccgaagaagcacaaaaagaactggaagaaaacaacgagaaaatcaaaaatgcacagggcctgcagtattataacccggaagaagaaatgctttgcgaagtggaaatcaccaaaaactatgaagccacctatgtgattaaacagagccagggtattctgtgggcaggcaaaaaaggcatgaaagccgctaaaaccaaaagcaccgtgaaaaatctgatgctgctgctgcaacatgtggcaaccgaaagcattacccgtgttggtaaatgtccgacctttaaagttccgtttaccaaagaacaggtgatgtgggaaatgcagaaaggttggtattatagttggctgccggaaattgtttatacccatcaggttgttcatgatgactggcgtatgaaactggttgaagaaccgaccagcggtattaccatttataccggtggtggtaaacagaatggtgaaggtattgcagcctatgttaccagcaatggtcgtaccaaacagaaacgtctgggtccggttacacatcaggtggcagaacgtatggcaattcagatggcactggaagatacccgtgataaacgggttaatattgtgaccgatagctattattgttggaaaaacattaccgaaggtctgggtctggaaggtccgcagagcccgtggtggccgattattcagaatattcacgaaaaagaaatcgtgtactttgcatgggttccaggtcataaaggtatttgtggtaatcagctggcagatgaagcagccaaaatcaaagaagagatc

SEQ ID NO: 14 - protein, 558 aa, Artificial Sequence
  Expression from a synthetic gene
MAQLSKEIKFRKIELKEGTMGPKIPQWPLTKEKLEGAKEIVQRLLSEGKISEASDNNPYNSPIFVIKKRSGKWRLLQDLRELNKTVQVGTEISRGLPHPGGLIKCKHMTVLDIGDAYFTIPLDPEFRPYTAFTIPSINHQEPDKRYVWNCLPQGFVLSPYIYQKTLQEILQPFRERYPEVQLYQYMDDLFVGSNGSKKQHKELIIELRAILLEKGFETPDDKLQEVPPYSWLGYQLCPENWKVQKMQLDMVKNPTLNDVQKLVGKINWASQGVPGLTVKHIAATTKGCLELNQKVIWTEEAQKELEENNEKIKNAQGLQYYNPEEEMLCEVEITKNYEATYVIKQSQGILWAGKKGMKAAKTKSTVKNLMLLLQHVATESITRVGKCPTFKVPFTKEQVMWEMQKGWYYSWLPEIVYTHQVVHDDWRMKLVEEPTSGITIYTGGGKQNGEGIAAYVTSNGRTKQKRLGPVTHQVAERMAIQMALEDTRDKRVNIVTDSYYCWKNITEGLGLEGPQSPWWPIIQNIHEKEIVYFAWVPGHKGICGNQLADEAAKIKEEI